European Patent Application EP 4 238 983 A1, published September 6, 2023. Title: Vaccine composition for preventing or treating infection of SARS-CoV-2. Applicant: SK bioscience Co., Ltd. The sequence listing filed with the application follows.

SEQUENCE LISTING (28 sequences)

SEQ ID NO: 1 - protein, 15 aa, Artificial Sequence
  Tetanus toxoid P2 epitope  peptide
QYIKANSKFIGITEL

SEQ ID NO: 2 - protein, 673 aa, Artificial Sequence
  the fragment from 14 to 686 amino acids of S protein of Sars-cov-2
QCVNLTTRTQLPPAYTNSFTRGVYYPDKVFRSSVLHSTQDLFLPFFSNVTWFHAIHVSGTNGTKRFDNPVLPFNDGVYFASTEKSNIIRGWIFGTTLDSKTQSLLIVNNATNVVIKVCEFQFCNDPFLGVYYHKNNKSWMESEFRVYSSANNCTFEYVSQPFLMDLEGKQGNFKNLREFVFKNIDGYFKIYSKHTPINLVRDLPQGFSALEPLVDLPIGINITRFQTLLALHRSYLTPGDSSSGWTAGAAAYYVGYLQPRTFLLKYNENGTITDAVDCALDPLSETKCTLKSFTVEKGIYQTSNFRVQPTESIVRFPNITNLCPFGEVFNATRFASVYAWNRKRISNCVADYSVLYNSASFSTFKCYGVSPTKLNDLCFTNVYADSFVIRGDEVRQIAPGQTGKIADYNYKLPDDFTGCVIAWNSNNLDSKVGGNYNYLYRLFRKSNLKPFERDISTEIYQAGSTPCNGVEGFNCYFPLQSYGFQPTNGVGYQPYRVVVLSFELLHAPATVCGPKKSTNLVKNKCVNFNFNGLTGTGVLTESNKKFLPFQQFGRDIADTTDAVRDPQTLEILDITPCSFGGVSVITPGTNTSNQVAVLYQDVNCTEVPVAIHADQLTPTWRVYSTGSNVFQTRAGCLIGAEHVNNSYECDIPIGAGICASYQTQTNSPRRARS

SEQ ID NO: 3 - protein, 269 aa, Artificial Sequence
  the fragment from 323 to 591 amino acids of S protein of Sars-cov-2
TESIVRFPNITNLCPFGEVFNATRFASVYAWNRKRISNCVADYSVLYNSASFSTFKCYGVSPTKLNDLCFTNVYADSFVIRGDEVRQIAPGQTGKIADYNYKLPDDFTGCVIAWNSNNLDSKVGGNYNYLYRLFRKSNLKPFERDISTEIYQAGSTPCNGVEGFNCYFPLQSYGFQPTNGVGYQPYRVVVLSFELLHAPATVCGPKKSTNLVKNKCVNFNFNGLTGTGVLTESNKKFLPFQQFGRDIADTTDAVRDPQTLEILDITPCS

SEQ ID NO: 4 - protein, 217 aa, Artificial Sequence
  the fragment from 321 to 537 amino acids of S protein of Sars-cov-2
QPTESIVRFPNITNLCPFGEVFNATRFASVYAWNRKRISNCVADYSVLYNSASFSTFKCYGVSPTKLNDLCFTNVYADSFVIRGDEVRQIAPGQTGKIADYNYKLPDDFTGCVIAWNSNNLDSKVGGNYNYLYRLFRKSNLKPFERDISTEIYQAGSTPCNGVEGFNCYFPLQSYGFQPTNGVGYQPYRVVVLSFELLHAPATVCGPKKSTNLVKNK

SEQ ID NO: 5 - protein, 181 aa, Artificial Sequence
  the fragment from 336 to 516 amino acids of S protein of Sars-cov-2
CPFGEVFNATRFASVYAWNRKRISNCVADYSVLYNSASFSTFKCYGVSPTKLNDLCFTNVYADSFVIRGDEVRQIAPGQTGKIADYNYKLPDDFTGCVIAWNSNNLDSKVGGNYNYLYRLFRKSNLKPFERDISTEIYQAGSTPCNGVEGFNCYFPLQSYGFQPTNGVGYQPYRVVVLSFE

SEQ ID NO: 6 - protein, 694 aa, Artificial Sequence
  SK-E-S1-P2
MQYIKANSKFIGITELGSGSGQCVNLTTRTQLPPAYTNSFTRGVYYPDKVFRSSVLHSTQDLFLPFFSNVTWFHAIHVSGTNGTKRFDNPVLPFNDGVYFASTEKSNIIRGWIFGTTLDSKTQSLLIVNNATNVVIKVCEFQFCNDPFLGVYYHKNNKSWMESEFRVYSSANNCTFEYVSQPFLMDLEGKQGNFKNLREFVFKNIDGYFKIYSKHTPINLVRDLPQGFSALEPLVDLPIGINITRFQTLLALHRSYLTPGDSSSGWTAGAAAYYVGYLQPRTFLLKYNENGTITDAVDCALDPLSETKCTLKSFTVEKGIYQTSNFRVQPTESIVRFPNITNLCPFGEVFNATRFASVYAWNRKRISNCVADYSVLYNSASFSTFKCYGVSPTKLNDLCFTNVYADSFVIRGDEVRQIAPGQTGKIADYNYKLPDDFTGCVIAWNSNNLDSKVGGNYNYLYRLFRKSNLKPFERDISTEIYQAGSTPCNGVEGFNCYFPLQSYGFQPTNGVGYQPYRVVVLSFELLHAPATVCGPKKSTNLVKNKCVNFNFNGLTGTGVLTESNKKFLPFQQFGRDIADTTDAVRDPQTLEILDITPCSFGGVSVITPGTNTSNQVAVLYQDVNCTEVPVAIHADQLTPTWRVYSTGSNVFQTRAGCLIGAEHVNNSYECDIPIGAGICASYQTQTNSPRRARS

SEQ ID NO: 7 - protein, 290 aa, Artificial Sequence
  SK-E-S1-T1-P2
MQYIKANSKFIGITELGSGSGTESIVRFPNITNLCPFGEVFNATRFASVYAWNRKRISNCVADYSVLYNSASFSTFKCYGVSPTKLNDLCFTNVYADSFVIRGDEVRQIAPGQTGKIADYNYKLPDDFTGCVIAWNSNNLDSKVGGNYNYLYRLFRKSNLKPFERDISTEIYQAGSTPCNGVEGFNCYFPLQSYGFQPTNGVGYQPYRVVVLSFELLHAPATVCGPKKSTNLVKNKCVNFNFNGLTGTGVLTESNKKFLPFQQFGRDIADTTDAVRDPQTLEILDITPCS

SEQ ID NO: 8 - protein, 238 aa, Artificial Sequence
  SK-E-RBD-Ex3-P2
MQYIKANSKFIGITELGSGSGQPTESIVRFPNITNLCPFGEVFNATRFASVYAWNRKRISNCVADYSVLYNSASFSTFKCYGVSPTKLNDLCFTNVYADSFVIRGDEVRQIAPGQTGKIADYNYKLPDDFTGCVIAWNSNNLDSKVGGNYNYLYRLFRKSNLKPFERDISTEIYQAGSTPCNGVEGFNCYFPLQSYGFQPTNGVGYQPYRVVVLSFELLHAPATVCGPKKSTNLVKNK

SEQ ID NO: 9 - protein, 202 aa, Artificial Sequence
  SK-E-RBD-P2
MQYIKANSKFIGITELGSGSGCPFGEVFNATRFASVYAWNRKRISNCVADYSVLYNSASFSTFKCYGVSPTKLNDLCFTNVYADSFVIRGDEVRQIAPGQTGKIADYNYKLPDDFTGCVIAWNSNNLDSKVGGNYNYLYRLFRKSNLKPFERDISTEIYQAGSTPCNGVEGFNCYFPLQSYGFQPTNGVGYQPYRVVVLSFE

SEQ ID NO: 10 - protein, 270 aa, Artificial Sequence
  SK-E-RBD-Ex3-foldon-P2
MQYIKANSKFIGITELGSGSGQPTESIVRFPNITNLCPFGEVFNATRFASVYAWNRKRISNCVADYSVLYNSASFSTFKCYGVSPTKLNDLCFTNVYADSFVIRGDEVRQIAPGQTGKIADYNYKLPDDFTGCVIAWNSNNLDSKVGGNYNYLYRLFRKSNLKPFERDISTEIYQAGSTPCNGVEGFNCYFPLQSYGFQPTNGVGYQPYRVVVLSFELLHAPATVCGPKKSTNLVKNKGSGGSGYIPEAPRDGQAYVRKDGEWVLLSTFL

SEQ ID NO: 11 - DNA, 2085 bp, Artificial Sequence
  the optimized codon of SK-E-S1-P2
atgcagtatataaaagcaaattctaaatttataggtataactgaactaggctccggctcaggccagtgtgttaatcttacaaccagaactcaattaccccctgcatacactaattctttcacacgtggtgtttattaccctgacaaagttttcagatcctcagttttacattcaactcaggacttgttcttacctttcttttccaatgttacttggttccatgctatacatgtctctgggaccaatggtactaagaggtttgataaccctgtcctaccatttaatgatggtgtttattttgcttccactgagaagtctaacataataagaggctggatttttggtactactttagattcgaagacccagtccctacttattgttaataacgctactaatgttgttattaaagtctgtgaatttcaattttgtaatgatccatttttgggtgtttattaccacaaaaacaacaaaagttggatggaaagtgagttcagagtttattctagtgcgaataattgcacttttgaatatgtctctcagccttttcttatggaccttgaaggaaaacagggtaatttcaaaaatcttagggaatttgtgtttaagaatattgatggttattttaaaatatattctaagcacacgcctattaatttagtgcgtgatctccctcagggtttttcggctttagaaccattggtagatttgccaataggtattaacatcactaggtttcaaactttacttgctttacatagaagttatttgactcctggtgattcttcttcaggttggacagctggtgctgcagcttattatgtgggttatcttcaacctaggacttttctattaaaatataatgaaaatggaaccattacagatgctgtagactgtgcacttgaccctctctcagaaacaaagtgtacgttgaaatccttcactgtagaaaaaggaatctatcaaacttctaactttagagtccaaccaacagaatctattgttagatttcctaatattacaaacttgtgcccttttggtgaagtttttaacgccaccagatttgcatctgtttatgcttggaacaggaagagaatcagcaactgtgttgctgattattctgtcctatataattccgcatcattttccacttttaagtgttatggagtgtctcctactaaattaaatgatctctgctttactaatgtctatgcagattcatttgtaattagaggtgatgaagtcagacaaatcgctccagggcaaactggaaagattgctgattataattataaattaccagatgattttacaggctgcgttatagcttggaattctaacaatcttgattctaaggttggtggtaattataattacctgtatagattgtttaggaagtctaatctcaaaccttttgagagagatatttcaactgaaatctatcaggccggtagcacaccttgtaatggtgttgaaggttttaattgttactttcctttacaatcttatggtttccaacccactaatggtgttggttaccaaccatacagagtagtagtactttcttttgaacttctacatgcaccagcaactgtttgtggacctaaaaagtctactaatttggttaaaaacaaatgtgtcaatttcaacttcaatggtttaacaggcacaggtgttcttactgagtctaacaaaaagtttctgcctttccaacaatttggcagagacattgctgacactactgatgctgtccgtgatccacagacacttgagattcttgacattacaccatgttcttttggtggtgtcagtgttataacaccaggaacaaatacttctaaccaggttgctgttctttatcaggatgttaactgcacagaagtccctgttgctattcatgcagatcaacttactcctacttggcgtgtttattctacaggttctaatgtttttcaaacacgtgcaggctgtttaataggggctgaacatgtcaacaactcttatgagtgtgacatacccattggtgcaggtatatgcgctagttatcagactcagactaattctcctcggcgggcacgtagttga

SEQ ID NO: 12 - DNA, 873 bp, Artificial Sequence
  the optimized codon of SK-E-S1-T1-P2
atgcagtatataaaagcaaattctaaatttataggtataactgaactaggctccggctcaggcaccgaaagcattgttcgtttcccgaacatcaccaacctgtgcccgtttggcgaggtgttcaacgcgacccgtttcgcgagcgtttatgcgtggaaccgtaaacgtatcagcaactgcgttgcggattatagcgtgctgtacaacagcgcgagcttcagcacctttaagtgctatggtgttagcccgaccaaactgaacgacctgtgctttaccaacgtttacgcggatagcttcgtgattcgtggcgacgaagttcgtcagatcgcgccgggtcaaaccggcaagattgcggattacaactataaactgccggacgatttcaccggttgcgtgattgcgtggaacagcaacaacctggacagcaaggttggtggcaactacaactatctgtaccgtctgtttcgtaagagcaacctgaaaccgttcgagcgtgatattagcaccgaaatctaccaggcgggtagcaccccgtgcaacggtgtggaaggctttaactgctatttcccgctgcagagctacggctttcaaccgaccaacggtgttggctatcaaccgtaccgtgtggttgttctgagcttcgagctgctgcatgcgccggcgaccgtttgcggtccgaagaaaagcaccaacctggttaagaacaaatgcgtgaacttcaactttaacggcctgaccggcaccggtgtgctgaccgaaagcaacaagaaattcctgccgtttcagcaattcggtcgtgacatcgcggataccaccgacgcggttcgtgatccgcagaccctggagattctggacatcaccccgtgcagctaa

SEQ ID NO: 13 - DNA, 714 bp, Artificial Sequence
  the optimized codon of SK-E-RBD-Ex3-P2
atgcagtatataaaagcaaattctaaatttataggtataactgaactaggctccggctcaggccaaccgaccgaaagcattgttcgtttcccgaacatcaccaacctgtgcccgtttggcgaggtgttcaacgcgacccgtttcgcgagcgtttatgcgtggaaccgtaaacgtatcagcaactgcgttgcggattatagcgtgctgtacaacagcgcgagcttcagcacctttaagtgctatggtgttagcccgaccaaactgaacgacctgtgctttaccaacgtttacgcggatagcttcgtgattcgtggcgacgaagttcgtcagatcgcgccgggtcaaaccggcaagattgcggattacaactataaactgccggacgatttcaccggttgcgtgattgcgtggaacagcaacaacctggacagcaaggttggtggcaactacaactatctgtaccgtctgtttcgtaagagcaacctgaaaccgttcgagcgtgatattagcaccgaaatctaccaggcgggtagcaccccgtgcaacggtgtggaaggctttaactgctatttcccgctgcagagctacggctttcaaccgaccaacggtgttggctatcaaccgtaccgtgtggttgttctgagcttcgagctgctgcatgcgccggcgaccgtttgcggtccgaagaaaagcaccaacctggttaagaacaaa

SEQ ID NO: 14 - DNA, 609 bp, Artificial Sequence
  the optimized codon of SK-E-RBD-P2
atgcagtatataaaagcaaattctaaatttataggtataactgaactaggctccggctcaggctgcccttttggtgaagtttttaacgccaccagatttgcatctgtttatgcttggaacaggaagagaatcagcaactgtgttgctgattattctgtcctatataattccgcatcattttccacttttaagtgttatggagtgtctcctactaaattaaatgatctctgctttactaatgtctatgcagattcatttgtaattagaggtgatgaagtcagacaaatcgctccagggcaaactggaaagattgctgattataattataaattaccagatgattttacaggctgcgttatagcttggaattctaacaatcttgattctaaggttggtggtaattataattacctgtatagattgtttaggaagtctaatctcaaaccttttgagagagatatttcaactgaaatctatcaggccggtagcacaccttgtaatggtgttgaaggttttaattgttactttcctttacaatcttatggtttccaacccactaatggtgttggttaccaaccatacagagtagtagtactttcttttgaataa

SEQ ID NO: 15 - DNA, 810 bp, Artificial Sequence
  the optimized codon of SK-E-RBD-Ex3-foldon-P2
atgcagtatataaaagcaaattctaaatttataggtataactgaactaggctccggctcaggccaaccgaccgaaagcattgttcgtttcccgaacatcaccaacctgtgcccgtttggcgaggtgttcaacgcgacccgtttcgcgagcgtttatgcgtggaaccgtaaacgtatcagcaactgcgttgcggattatagcgtgctgtacaacagcgcgagcttcagcacctttaagtgctatggtgttagcccgaccaaactgaacgacctgtgctttaccaacgtttacgcggatagcttcgtgattcgtggcgacgaagttcgtcagatcgcgccgggtcaaaccggcaagattgcggattacaactataaactgccggacgatttcaccggttgcgtgattgcgtggaacagcaacaacctggacagcaaggttggtggcaactacaactatctgtaccgtctgtttcgtaagagcaacctgaaaccgttcgagcgtgatattagcaccgaaatctaccaggcgggtagcaccccgtgcaacggtgtggaaggctttaactgctatttcccgctgcagagctacggctttcaaccgaccaacggtgttggctatcaaccgtaccgtgtggttgttctgagcttcgagctgctgcatgcgccggcgaccgtttgcggtccgaagaaaagcaccaacctggttaagaacaaaggtagcggtggcagcggttacatccctgaagctccccgcgacggacaggcctacgtccgtaaggacggagaatgggtactcctgtctacgttcctg

SEQ ID NO: 16 - protein, 439 aa, Artificial Sequence
  SK-E-N
MQYIKANSKFIGITELGSGSGSDNGPQNQRNAPRITFGGPSDSTGSNQNGERSGARSKQRRPQGLPNNTASWFTALTQHGKEDLKFPRGQGVPINTNSSPDDQIGYYRRATRRIRGGDGKMKDLSPRWYFYYLGTGPEAGLPYGANKDGIIWVATEGALNTPKDHIGTRNPANNAAIVLQLPQGTTLPKGFYAEGSRGGSQASSRSSSRSRNSSRNSTPGSSRGTSPARMAGNGGDAALALLLLDRLNQLESKMSGKGQQQQGQTVTKKSAAEASKKPRQKRTATKAYNVTQAFGRRGPEQTQGNFGDQELIRQGTDYKHWPQIAQFAPSASAFFGMSRIGMEVTPSGTWLTYTGAIKLDDKDPNFKDQVILLNKHIDAYKTFPPTEPKKDKKKKADETQALPQRQKKQQTVTLLPAADLDDFSKQLQQSMSSADSTQA

SEQ ID NO: 17 - DNA, 2022 bp, Artificial Sequence
  the nucleotide sequences encoding the fragment from 14 to 686 amino acids of S protein
caatgcgttaatctgaccacccgcacccaactgccgccggcgtacaccaatagcttcacccgtggcgtttactacccggacaaggttttccgtagcagcgtgctgcacagcacccaggacctgtttctgccgttctttagcaacgtgacctggttccacgcgatccacgttagcggcaccaacggcaccaaacgttttgataacccggtgctgccgtttaacgacggtgtttacttcgcgagcaccgaaaagagcaacatcattcgtggttggattttcggcaccaccctggatagcaaaacccagagcctgctgatcgtgaacaacgcgaccaacgtggttattaaggtttgcgagttccaattttgcaacgacccgtttctgggcgtgtactatcacaagaacaacaaaagctggatggagagcgagttccgtgtgtatagcagcgcgaacaactgcacctttgagtacgttagccagccgttcctgatggatctggaaggcaagcaaggcaactttaaaaacctgcgtgagttcgttttcaagaacatcgacggttacttcaaaatctacagcaaacacaccccgatcaacctggtgcgtgatctgccgcagggttttagcgcgctggaaccgctggttgacctgccgatcggcattaacatcacccgtttccaaaccctgctggcgctgcaccgtagctacctgaccccgggtgacagcagcagcggttggaccgcgggtgctgcggcgtactatgtgggttatctgcagccgcgtacctttctgctgaaatacaacgagaacggcaccatcaccgatgcggtggattgcgcgctggacccgctgagcgaaaccaagtgcaccctgaagagcttcaccgttgagaagggtatttaccagaccagcaactttcgtgtgcaaccgaccgaaagcattgttcgtttcccgaacatcaccaacctgtgcccgtttggcgaggtgttcaacgcgacccgtttcgcgagcgtttatgcgtggaaccgtaaacgtatcagcaactgcgttgcggattatagcgtgctgtacaacagcgcgagcttcagcacctttaagtgctatggtgttagcccgaccaaactgaacgacctgtgctttaccaacgtttacgcggatagcttcgtgattcgtggcgacgaagttcgtcagatcgcgccgggtcaaaccggcaagattgcggattacaactataaactgccggacgatttcaccggttgcgtgattgcgtggaacagcaacaacctggacagcaaggttggtggcaactacaactatctgtaccgtctgtttcgtaagagcaacctgaaaccgttcgagcgtgatattagcaccgaaatctaccaggcgggtagcaccccgtgcaacggtgtggaaggctttaactgctatttcccgctgcagagctacggctttcaaccgaccaacggtgttggctatcaaccgtaccgtgtggttgttctgagcttcgagctgctgcatgcgccggcgaccgtttgcggtccgaagaaaagcaccaacctggttaagaacaaatgcgtgaacttcaactttaacggcctgaccggcaccggtgtgctgaccgaaagcaacaagaaattcctgccgtttcagcaattcggtcgtgacatcgcggataccaccgacgcggttcgtgatccgcagaccctggagattctggacatcaccccgtgcagctttggtggcgttagcgtgatcaccccgggcaccaacaccagcaaccaggttgcggtgctgtatcaagatgtgaactgcaccgaggttccggtggcgattcatgcggaccagctgaccccgacctggcgtgtgtacagcaccggtagcaacgttttccaaacccgtgcgggttgcctgattggtgcggagcacgttaacaacagctatgaatgcgacattccgatcggcgcgggtatttgcgcgagctatcagacccagaccaacagcccgcgtcgtgcgcgtagctaa

SEQ ID NO: 18 - DNA, 807 bp, Artificial Sequence
  the nucleotide sequences encoding the fragment from 323 to 591 amino acids of S protein
accgaaagcattgttcgtttcccgaacatcaccaacctgtgcccgtttggcgaggtgttcaacgcgacccgtttcgcgagcgtttatgcgtggaaccgtaaacgtatcagcaactgcgttgcggattatagcgtgctgtacaacagcgcgagcttcagcacctttaagtgctatggtgttagcccgaccaaactgaacgacctgtgctttaccaacgtttacgcggatagcttcgtgattcgtggcgacgaagttcgtcagatcgcgccgggtcaaaccggcaagattgcggattacaactataaactgccggacgatttcaccggttgcgtgattgcgtggaacagcaacaacctggacagcaaggttggtggcaactacaactatctgtaccgtctgtttcgtaagagcaacctgaaaccgttcgagcgtgatattagcaccgaaatctaccaggcgggtagcaccccgtgcaacggtgtggaaggctttaactgctatttcccgctgcagagctacggctttcaaccgaccaacggtgttggctatcaaccgtaccgtgtggttgttctgagcttcgagctgctgcatgcgccggcgaccgtttgcggtccgaagaaaagcaccaacctggttaagaacaaatgcgtgaacttcaactttaacggcctgaccggcaccggtgtgctgaccgaaagcaacaagaaattcctgccgtttcagcaattcggtcgtgacatcgcggataccaccgacgcggttcgtgatccgcagaccctggagattctggacatcaccccgtgcagc

SEQ ID NO: 19 - DNA, 651 bp, Artificial Sequence
  the nucleotide sequences encoding the fragment from 321 to 537 amino acids of S protein
caaccgaccgaaagcattgttcgtttcccgaacatcaccaacctgtgcccgtttggcgaggtgttcaacgcgacccgtttcgcgagcgtttatgcgtggaaccgtaaacgtatcagcaactgcgttgcggattatagcgtgctgtacaacagcgcgagcttcagcacctttaagtgctatggtgttagcccgaccaaactgaacgacctgtgctttaccaacgtttacgcggatagcttcgtgattcgtggcgacgaagttcgtcagatcgcgccgggtcaaaccggcaagattgcggattacaactataaactgccggacgatttcaccggttgcgtgattgcgtggaacagcaacaacctggacagcaaggttggtggcaactacaactatctgtaccgtctgtttcgtaagagcaacctgaaaccgttcgagcgtgatattagcaccgaaatctaccaggcgggtagcaccccgtgcaacggtgtggaaggctttaactgctatttcccgctgcagagctacggctttcaaccgaccaacggtgttggctatcaaccgtaccgtgtggttgttctgagcttcgagctgctgcatgcgccggcgaccgtttgcggtccgaagaaaagcaccaacctggttaagaacaaa

SEQ ID NO: 20 - DNA, 543 bp, Artificial Sequence
  the nucleotide sequences encoding the fragment from 336 to 516 amino acids of S protein
tgcccgtttggcgaggtgttcaacgcgacccgtttcgcgagcgtttatgcgtggaaccgtaaacgtatcagcaactgcgttgcggattatagcgtgctgtacaacagcgcgagcttcagcacctttaagtgctatggtgttagcccgaccaaactgaacgacctgtgctttaccaacgtttacgcggatagcttcgtgattcgtggcgacgaagttcgtcagatcgcgccgggtcaaaccggcaagattgcggattacaactataaactgccggacgatttcaccggttgcgtgattgcgtggaacagcaacaacctggacagcaaggttggtggcaactacaactatctgtaccgtctgtttcgtaagagcaacctgaaaccgttcgagcgtgatattagcaccgaaatctaccaggcgggtagcaccccgtgcaacggtgtggaaggctttaactgctatttcccgctgcagagctacggctttcaaccgaccaacggtgttggctatcaaccgtaccgtgtggttgttctgagcttcgag

SEQ ID NO: 21 - protein, 27 aa, Artificial Sequence
  foldon domain
GYIPEAPRDGQAYVRKDGEWVLLSTFL

SEQ ID NO: 22 - DNA, 1260 bp, Artificial Sequence
  the optimized codon of SK-E-N
atgtctgataatggaccccaaaatcagcgaaatgcaccccgcattacgtttggtggaccctcagattcaactggcagtaaccagaatggagaacgcagtggggcgcgatcaaaacaacgtcggccccaaggtttacccaataatactgcgtcttggttcaccgctctcactcaacatggcaaggaagaccttaaattccctcgaggacaaggcgttccaattaacaccaatagcagtccagatgaccaaattggctactaccgaagagctaccagacgaattcgtggtggtgacggtaaaatgaaagatctcagtccaagatggtatttctactacctaggaactgggccagaagctggacttccctatggtgctaacaaagacggcatcatttgggttgcaactgagggagccttgaatacaccaaaagatcacattggcacccgcaatcctgctaacaatgctgcaatcgtgctacaacttcctcaaggaacaacattgccaaaaggcttctacgcagaagggagcagaggcggcagtcaagcctcttctcgttcctcatcacgtagtcgcaacagttcaagaaattcaactccaggcagcagtaggggaacttctcctgctagaatggctggcaatggcggtgatgctgctcttgctttgctgctgcttgacagattgaaccagcttgagagcaaaatgtctggtaaaggccaacaacaacaaggccaaactgtcactaagaaatctgctgctgaggcttctaagaagcctcggcaaaaacgtactgccactaaagcatacaatgtaacacaagctttcggcagacgtggtccagaacaaacccaaggaaattttggggaccaggaactaatcagacaaggaactgattacaaacattggccgcaaattgcacaatttgcccccagcgcttcagcgttcttcggaatgtcgcgcattggcatggaagtcacaccttcgggaacgtggttgacctacacaggtgccatcaaattggatgacaaagatccaaatttcaaagatcaagtcattttgctgaataagcatattgacgcatacaaaacattcccaccaacagagcctaaaaaggacaaaaagaagaaggctgatgaaactcaagccttaccgcagagacagaagaaacagcaaactgtgactcttcttcctgctgcagatttggatgatttctccaaacaattgcaacaatccatgagcagtgctgactcaactcaggcctaa

SEQ ID NO: 23 - protein, 5 aa, Artificial Sequence
  GSGSG linker
GSGSG

SEQ ID NO: 24 - protein, 4 aa, Artificial Sequence
  GSSG linker
GSSG

SEQ ID NO: 25 - protein, 5 aa, Artificial Sequence
  GSGGS linker
GSGGS

SEQ ID NO: 26 - protein, 4 aa, Artificial Sequence
  GSGS linker
GSGS

SEQ ID NO: 27 - protein, 6 aa, Artificial Sequence
  GSGSSG linker
GSGSSG

SEQ ID NO: 28 - protein, 21 aa, Artificial Sequence
  pelB leader sequence
KYLLPTAAAGLLLLAAQPAMA